European Patent Application EP 4 682 170 A1, published January 21, 2026. Title: Novel CD3 Binding Antibodies and Multispecific Antibodies Including The Same. Applicant: MUSTBIO Co., Ltd. The sequence listing filed with the application follows.

SEQUENCE LISTING (42 sequences)

SEQ ID NO: 1 - protein, 122 aa, synthetic construct
EVQLVESGGGLVQPGGSLRLSCAASGFSFTGYTMNWVRQAPGKGLEWVALINPYKGVTTYADSVKGRFTISRDNSKNTAYLQMNSLRAEDTAVYYCARSGYYGDSDWYFDVWGQGTLVTVSS

SEQ ID NO: 2 - protein, 122 aa, synthetic construct
EVQLVESGGGLVQPGGSLRLSCAASGFSFTGYTMNWVRQAPGKGLEWVALINPYKGVTTYADSVKGRFTISRDNSKNTLYLQMNSLRAEDTAVYYCARSGYYGDSDWYFDVWGQGTLVTVSS

SEQ ID NO: 3 - protein, 122 aa, synthetic construct
EVQLVESGGGLVQPGGSLRLSCAASGFSFTGYTMNWVRQAPGKCLEWVALINPYKGVTTYADSVKGRFTISRDNSKNTLYLQMNSLRAEDTAVYYCARSGYYGDSDWYFDVWGQGTLVTVSS

SEQ ID NO: 4 - protein, 122 aa, synthetic construct
EVQLVESGGGLVQPGGSLRLSCAASGFSFTGYTMNWVRQAPGKGLEWVALINPYKGVTTYADSVKGRFTISADNSKNTLYLQMNSLRAEDTAVYYCARSGYYGDSDWYFDVWGQGTLVTVSS

SEQ ID NO: 5 - protein, 122 aa, synthetic construct
EVQLVESGGGLVQPGGSLRLSCAASGFSFTGYTMNWVRQAPGKCLEWVALINPYKGVTTYADSVKGRFTISADNSKNTLYLQMNSLRAEDTAVYYCARSGYYGDSDWYFDVWGQGTLVTVSS

SEQ ID NO: 6 - protein, 122 aa, synthetic construct
EVQLVESGGGLVQPGGSLRLSCAASGFSFTGYTMNWVRQAPGKGLEWVALINPYKGVTTYADSVKGRFTISDDNSKNTLYLQMNSLRAEDTAVYYCARSGYYGDSDWYFDVWGQGTLVTVSS

SEQ ID NO: 7 - protein, 122 aa, synthetic construct
EVQLVESGGGLVQPGGSLRLSCAASGFSFTGYTMNWVRQAPGKGLEWVALINPYKGVTTYADSVKGRFTISQDNSKNTLYLQMNSLRAEDTAVYYCARSGYYGDSDWYFDVWGQGTLVTVSS

SEQ ID NO: 8 - protein, 109 aa, synthetic construct
DIQMTQSPSSLSASVGDRVTITCRASQDIRNYLNWYQQKPGKAPKLLIYYTSRLESGVPSRFSGSGSGTDYTLTISSLQPEDFATYYCQQGNTLPWTFGQGTKVEIKRT

SEQ ID NO: 9 - protein, 109 aa, synthetic construct
DIQMTQSPSSLSASVGDRVTITCRASQDIRNYLNWYQQKPGKAPKLLIYYTSSLESGVPSRFSGSGSGTDYTLTISSLQPEDFATYYCQQGNTLPWTFGQGTKVEIKRT

SEQ ID NO: 10 - protein, 109 aa, synthetic construct
DIQMTQSPSSLSASVGDRVTITCRASQDIRNYLNWYQQKPGKAPKLLIYYTSSLESGVPSRFSGSGSGTDYTLTISSLQPEDFATYYCQQGNTLPWTFGCGTKVEIKRT

SEQ ID NO: 11 - protein, 119 aa, synthetic construct
DIKLQQSGAELARPGASVKMSCKTSGYTFTRYTMHWVKQRPGQGLEWIGYINPSRGYTNYNQKFKDKATLTTDKSSSTAYMQLSSLTSEDSAVYYCARYYDDHYCLDYWGQGTTLTVSS

SEQ ID NO: 12 - protein, 106 aa, synthetic construct
DIQLTQSPAIMSASPGEKVTMTCRASSSVSYMNWYQQKSGTSPKRWIYDTSKVASGVPYRFSGSGSGTSYSLTISSMEAEDAATYYCQQWSSNPLTFGAGTKLELK

SEQ ID NO: 13 - protein, 18 aa, synthetic construct
VEGGSGGSGGSGGSGGVD

SEQ ID NO: 14 - protein, 15 aa, synthetic construct
GGGGSGGGGSGGGGS

SEQ ID NO: 15 - protein, 232 aa, synthetic construct
EPKSSDKTHTCPPCPAPELLGGPSVFLFPPKPKDTLMISRTPEVTCVVVDVSHEDPEVKFNWYVDGVEVHNAKTKPREEQYNSTYRVVSVLTVLHQDWLNGKEYKCKVSNKALPAPIEKTISKAKGQPREPQVYTLPPSRDELTKNQVSLTCLVKGFYPSDIAVEWESNGQPENNYKTTPPVLDSDGSFFLYSKLTVDKSRWQQGNVFSCSVMHEALHNHYTQKSLSLSPGK

SEQ ID NO: 16 - protein, 232 aa, synthetic construct
EPKSCDKTHTCPPCPAPEAAGGPSVFLFPPKPKDTLMISRTPEVTCVVVDVSHEDPEVKFNWYVDGVEVHNAKTKPREEQYNSTYRVVSVLTVLHQDWLNGKEYKCKVSNKALPAPIEKTISKAKGQPREPQVYTLPPSRDELTKNQVSLWCLVKGFYPSDIAVEWESNGQPENNYKTTPPVLDSDGSFFLYSKLTVDKSRWQQGNVFSCSVMHEALHNHYTQKSLSLSPGK

SEQ ID NO: 17 - protein, 232 aa, synthetic construct
EPKSSDKTHTCPPCPAPEAAGGPSVFLFPPKPKDTLMISRTPEVTCVVVDVSHEDPEVKFNWYVDGVEVHNAKTKPREEQYNSTYRVVSVLTVLHQDWLNGKEYKCKVSNKALPAPIEKTISKAKGQPREPQVYTGPPSRDELTKNQVSLSCAVKGFYPSDIAVEWESNGQPENNYKTTPPVLDSDGSFFLVSKLTVDKSRWQQGNVFSCSVMHEALHNHYTQKSLSLSPGK

SEQ ID NO: 18 - protein, 218 aa, synthetic construct
EVQLLESGGGLVQPGGSLRLSCAASGFTFSSYIMMWVRQAPGKGLEWVSSIYPSGGITFYADTVKGRFTISRDNSKNTLYLQMNSLRAEDTAVYYCARIKLGTVTTVDYWGQGTLVTVSSASTKGPSVFPLAPSSKSTSGGTAALGCLVKDYFPEPVTVSWNSGALTSGVHTFPAVLQSSGLYSLSSVVTVPSSSLGTQTYICNVNHKPSNTKVDKKV

SEQ ID NO: 19 - protein, 216 aa, synthetic construct
QSALTQPASVSGSPGQSITISCTGTSSDVGGYNYVSWYQQHPGKAPKLMIYDVSNRPSGVSNRFSGSKSGNTASLTISGLQAEDEADYYCSSYTSSSTRVFGTGTKVTVLGQPKANPTVTLFPPSSEELQANKATLVCLISDFYPGAVTVAWKADGSPVKAGVETTKPSKQSNNKYAASSYLSLTPEQWKSHRSYSCQVTHEGSTVEKTVAPTECS

SEQ ID NO: 20 - protein, 213 aa, synthetic construct
QVQLVQSGAEVKKPGASVKVSCKASGYTFTDYEMHWVRQAPGQGLEWMGALDPKTGDTAYSQKFKGRVTLTADKSTSTAYMELSSLTSEDTAVYYCTRFYSYTYWGQGTLVTVSSASTKGPSVFPLAPSSKSTSGGTAALGCLVKDYFPEPVTVSWNSGALTSGVHTFPAVLQSSGLYSLSSVVTVPSSSLGTQTYICNVNHKPSNTKVDKKV

SEQ ID NO: 21 - protein, 219 aa, synthetic construct
DVVMTQSPLSLPVTPGEPASISCRSSQSLVHSNRNTYLHWYLQKPGQSPQLLIYKVSNRFSGVPDRFSGSGSGTDFTLKISRVEAEDVGVYYCSQNTHVPPTFGQGTKLEIKRTVAAPSVFIFPPSDEQLKSGTASVVCLLNNFYPREAKVQWKVDNALQSGNSQESVTEQDSKDSTYSLSSTLTLSKADYEKHKVYACEVTHQGLSSPVTKSFNRGEC

SEQ ID NO: 22 - DNA, 366 bp, synthetic construct
  source 1..366: mol_type = other DNA
gaagtgcagctggtggaatctggcggaggattggttcagcctggcggctctctgagactgtcttgtgccgcctctggcttctctttcaccggctacaccatgaactgggtccgacaggctcctggcaaaggactggaatgggtcgccctgatcaacccctataagggcgtgaccacctacgccgactctgtgaagggcagattcaccatcagccgggacaactccaagaacaccgcctacctgcagatgaactccctgagagctgaggacaccgccgtgtactattgtgccagatccggctactacggcgactccgactggtactttgatgtgtggggacagggcaccctggtcacagtttctagt

SEQ ID NO: 23 - DNA, 366 bp, synthetic construct
  source 1..366: mol_type = other DNA
gaagtgcagctggtggaatctggcggaggattggttcagcctggcggctctctgagactgtcttgtgccgcctctggcttctctttcaccggctacaccatgaactgggtccgacaggctcctggcaaaggactggaatgggtcgccctgatcaacccctataagggcgtgaccacctacgccgactctgtgaagggcagattcaccatcagccgggacaactccaagaacaccctgtacctgcagatgaactccctgagagccgaggacaccgccgtgtactattgtgccagatccggctactacggcgactccgactggtactttgatgtgtggggacagggcaccctggtcacagtttctagt

SEQ ID NO: 24 - DNA, 366 bp, synthetic construct
  source 1..366: mol_type = other DNA
gaagtgcagctggtggaatctggcggaggattggttcagcctggcggctctctgagactgtcttgtgccgcctctggcttctctttcaccggctacaccatgaactgggtccgacaggctcctggcaaatgcctggaatgggtcgccctgatcaacccctataagggcgtgaccacctacgccgactctgtgaagggcagattcaccatcagccgggacaactccaagaacaccctgtacctgcagatgaactccctgagagccgaggacaccgccgtgtactattgtgccagatccggctactacggcgactccgactggtactttgatgtgtggggacagggcaccctggtcacagtttctagt

SEQ ID NO: 25 - DNA, 365 bp, synthetic construct
  source 1..365: mol_type = other DNA
gaagtgcagctggtggaatctggcggaggattggttcagcctggcggctctctgagactgtcttgtgccgcctctggcttctctttcaccggctacaccatgaactgggtccgacaggctcctggcaaagactggaatgggtcgccctgatcaacccctataagggcgtgaccacctacgccgactctgtgaagggcagattcaccatcagcgccgacaactccaagaacaccctgtacctgcagatgaactccctgagagccgaggacaccgccgtgtactattgtgccagatccggctactacggcgactccgactggtactttgatgtgtggggacagggcaccctggtcacagtttctagt

SEQ ID NO: 26 - DNA, 366 bp, synthetic construct
  source 1..366: mol_type = other DNA
gaagtgcagctggtggaatctggcggaggattggttcagcctggcggctctctgagactgtcttgtgccgcctctggcttctctttcaccggctacaccatgaactgggtccgacaggctcctggcaaatgcctggaatgggtcgccctgatcaacccctataagggcgtgaccacctacgccgactctgtgaagggcagattcaccatcagcgccgacaactccaagaacaccctgtacctgcagatgaactccctgagagccgaggacaccgccgtgtactattgtgccagatccggctactacggcgactccgactggtactttgatgtgtggggacagggcaccctggtcacagtttctagt

SEQ ID NO: 27 - DNA, 366 bp, synthetic construct
  source 1..366: mol_type = other DNA
gaagtgcagctggtggaatctggcggaggattggttcagcctggcggctctctgagactgtcttgtgccgcctctggcttctctttcaccggctacaccatgaactgggtccgacaggctcctggcaaaggactggaatgggtcgccctgatcaacccctataagggcgtgaccacctacgccgactctgtgaagggcagattcaccatcagcgacgacaactccaagaacaccctgtacctgcagatgaactccctgagagccgaggacaccgccgtgtactattgtgccagatccggctactacggcgactccgactggtactttgatgtgtggggacagggcaccctggtcacagtttctagt

SEQ ID NO: 28 - DNA, 366 bp, synthetic construct
  source 1..366: mol_type = other DNA
gaagtgcagctggtggaatctggcggaggattggttcagcctggcggctctctgagactgtcttgtgccgcctctggcttctctttcaccggctacaccatgaactgggtccgacaggctcctggcaaaggactggaatgggtcgccctgatcaacccctataagggcgtgaccacctacgccgactctgtgaagggcagattcaccatcagccaggacaactccaagaacaccctgtacctgcagatgaactccctgagagccgaggacaccgccgtgtactattgtgccagatccggctactacggcgactccgactggtactttgatgtgtggggacagggcaccctggtcacagtttctagt

SEQ ID NO: 29 - DNA, 342 bp, synthetic construct
  source 1..342: mol_type = other DNA
gatattcagatgacccagtctccttccagcctgtctgcctctgtgggcgacagagtgaccatcacctgtagagcctctcaggacatccggaactacctgaactggtatcagcagaagcccggcaaggcccctaagctgctgatctactacacctctagactggaatccggcgtgccctccagattttctggctctggatctggcaccgactacaccctgaccatcagttctctgcagcctgaggacttcgccacctactactgtcagcagggcaataccctgccttggacctttggccagggcaccaaggtggaaatcaagcggacagagcccaagtcctcc

SEQ ID NO: 30 - DNA, 327 bp, synthetic construct
  source 1..327: mol_type = other DNA
gatattcagatgacccagtctccttccagcctgtctgcctctgtgggcgacagagtgaccatcacctgtagagcctctcaggacatccggaactacctgaactggtatcagcagaagcccggcaaggcccctaagctgctgatctactacacctccagcctggaatccggcgtgccatccagattttctggatctggctctggcaccgactacaccctgaccattagttccctgcagcctgaggacttcgccacctactactgtcagcagggcaataccctgccttggacctttggccagggcaccaaggtggaaatcaagcggaca

SEQ ID NO: 31 - DNA, 327 bp, synthetic construct
  source 1..327: mol_type = other DNA
gatattcagatgacccagtctccttccagcctgtctgcctctgtgggcgacagagtgaccatcacctgtagagcctctcaggacatccggaactacctgaactggtatcagcagaagcccggcaaggcccctaagctgctgatctactacacctccagcctggaatccggcgtgccatccagattttctggatctggctctggcaccgactacaccctgaccattagttccctgcagcctgaggacttcgccacctactactgtcagcagggcaataccctgccttggacctttggctgcggcaccaaggtggaaatcaagcggaca

SEQ ID NO: 32 - DNA, 357 bp, synthetic construct
  source 1..357: mol_type = other DNA
gacatcaagctgcagcagtctggcgctgaattggccagacctggcgcctctgtgaagatgtcctgcaagacctccggctacaccttcaccagatacaccatgcactgggtcaagcagaggcctggacagggacttgagtggatcggctacatcaaccctagccggggctacaccaactacaaccagaagttcaaggacaaggctaccctgaccaccgacaagtcctcttccaccgcttacatgcagctgtccagcctgacctctgaggactctgccgtgtactactgcgcccggtactacgacgaccactactgtctggattactggggccagggcaccacactgacagtgtcatct

SEQ ID NO: 33 - DNA, 318 bp, synthetic construct
  source 1..318: mol_type = other DNA
gatattcagctgacccagtctcctgccatcatgtctgcttctcccggcgagaaagtgacaatgacctgcagagcctcctcctccgtgtcctacatgaactggtatcagcagaagtccggcacctctcctaagagatggatctacgacacctccaaggtggcctctggcgtgccatacagattttccggctctggatctggcaccagctactccctgaccatctcctctatggaagccgaggatgccgccacctactactgtcagcagtggtctagcaaccctctgacctttggcgctggcaccaagctggaactgaaa

SEQ ID NO: 34 - DNA, 54 bp, synthetic construct
  source 1..54: mol_type = other DNA
gttgaaggcggctctggcggaagcggaggtagcggaggatctggcggagtggac

SEQ ID NO: 35 - DNA, 45 bp, synthetic construct
  source 1..45: mol_type = other DNA
ggtggcggtggtagtggcggcggaggttcaggcggaggcggatct

SEQ ID NO: 36 - DNA, 696 bp, synthetic construct
  source 1..696: mol_type = other DNA
gagcccaagtcctccgacaagacccatacctgtcctccatgtcctgctccagaagctgctggcggaccctctgtgttcctgtttcctccaaagcctaaggacaccctgatgatctctcggacccctgaagtgacctgcgtggtggtggatgtgtctcacgaggacccagaagtgaagtttaattggtacgtggacggcgtggaagtgcacaacgccaagaccaagcctagagaggaacagtacaactccacctacagagtggtgtccgtgctgaccgtgctgcaccaggattggctgaacggcaaagagtacaagtgcaaggtgtccaacaaggccctgcctgctcctatcgaaaagaccatctccaaggctaagggccagcctcgggaacctcaggtttacacaggacctccatctcgggacgagctgaccaagaatcaggtgtccctgtcttgcgccgtgaagggcttctacccttccgacattgccgtggaatgggagtccaatggccagcctgagaacaactacaagaccacacctcctgtgctggactccgacggctcattcttcctggtgtccaagctgacagtggacaagtccagatggcagcagggaaacgtgttctcctgctctgtgatgcacgaggccctgcacaaccactacacacagaagtccctgagcctgtctccaggcaag

SEQ ID NO: 37 - DNA, 696 bp, synthetic construct
  source 1..696: mol_type = other DNA
gaacccaagtcctgcgacaagacccacacctgtcctccatgtcctgctccagaactgctcggcggtccctccgttttcctgtttccacctaagcctaaggacaccctgatgatctctcggacccctgaagtgacctgcgtggtggtggatgtgtctcacgaggacccagaagtgaagtttaattggtacgtggacggcgtggaagtgcacaacgccaagaccaagcctagagaggaacagtacaactccacctacagagtggtgtccgtgctgaccgtgctgcaccaggattggctgaacggcaaagagtacaagtgcaaggtgtccaacaaggccctgcctgctcctatcgaaaagaccatctccaaggctaagggccagcctcgggaacctcaggtttacacactgcctccatctcgggacgagctgaccaagaatcaggtgtccctgtggtgcctggttaagggcttctacccttccgacattgccgtggaatgggagtctaacggccagccagagaacaactacaagacaacccctcctgtgctggactccgacggctcattcttcctgtactccaagctgacagtggacaagtctcggtggcagcagggcaacgtgttctcctgttctgtgatgcacgaggccctgcacaaccactacacacagaagtccctgtctctgagccccggcaaa

SEQ ID NO: 38 - DNA, 696 bp, synthetic construct; identical to SEQ ID NO: 36
  source 1..696: mol_type = other DNA

SEQ ID NO: 39 - DNA, 654 bp, synthetic construct
  source 1..654: mol_type = other DNA
gaagtgcagctgctggaatctggcggaggattggttcagcctggcggctctctgagactgtcttgtgctgcctccggcttcaccttctccagctatatcatgatgtgggtccgacaggcccctggcaaaggactggaatgggtgtcctctatctacccctctggcggcatcaccttttacgccgataccgtgaagggcagattcaccatcagccgggacaactccaagaacaccctgtacctgcagatgaactccctgagagccgaggacaccgccgtgtactactgtgctagaatcaagctgggcaccgtgaccaccgtggattattggggacagggcacactggtcaccgtgtcctctgcttctaccaagggaccctctgtgttccctctggctccttccagcaagtctacatccggtggaaccgctgctctgggctgcctggtcaaggattactttcctgagcctgtgaccgtgtcttggaactctggtgctctgacctccggcgtgcacacatttccagctgtgctgcagtcctccggcctgtactctctgtcctctgtcgtgaccgtgccttctagctctctgggcacccagacctacatctgcaacgtgaaccacaagccttccaacaccaaggtggacaagaaggtg

SEQ ID NO: 40 - DNA, 648 bp, synthetic construct
  source 1..648: mol_type = other DNA
cagtccgctctgactcagcctgcttctgtgtctggctcccctggccagtctatcaccatctcttgtaccggcacctctagcgacgtcggcggctacaattacgtgtcctggtatcagcagcaccccggcaaggctcccaagctgatgatctacgacgtgtccaacagaccctccggcgtgtccaatcggttctctggctctaagtccggcaataccgcctctctgacaatcagtggactgcaggccgaggacgaggccgactactactgttcctcctacacctcctccagcaccagagtgtttggcaccggcaccaaagtgacagtgctgggccagcctaaggccaatcctaccgtgacactgttccctccatcctccgaggaactgcaggctaacaaggctaccctcgtgtgcctgatctccgatttttaccctggcgctgtgaccgtggcttggaaggctgatggatctcctgtgaaggccggcgtggaaaccaccaagcctagcaagcagtccaacaacaaatacgccgcctcctcctacctgtctctgacccctgaacagtggaagtcccaccggtcctactcttgccaagtgacccatgagggctccaccgtggaaaagacagtggcccctaccgagtgctcc

SEQ ID NO: 41 - DNA, 645 bp, synthetic construct
  source 1..645: mol_type = other DNA
cagtgtcaggtgcagctggtgcaatctggcgccgaagttaagaaacctggcgcctctgtgaaggtgtcctgcaaggcttctggctacacctttaccgactacgagatgcactgggtccgacaggctccaggacaaggattggaatggatgggcgctctggaccctaagaccggcgataccgcctacagccagaaattcaagggcagagtgaccctgaccgccgacaagtctacctccaccgcttacatggaactgtccagcctgacctctgaggacaccgccgtgtactactgcacccggttctactcttacacctactggggccagggcaccctggttacagtgtcctctgcttctaccaagggacccagcgttttccctctggctccatcctccaagtccacctctggtggaacagctgctctgggctgcctggtcaaggattactttcctgagcctgtgaccgtgtcctggaactctggtgctctgacatccggcgtgcacacctttccagctgtgctgcagtcctctggcctgtactctctgtcctctgtcgtgaccgtgccttctagctctctgggcacccagacctacatctgcaacgtgaaccacaagccttccaacaccaaagtggacaagaaggtg

SEQ ID NO: 42 - DNA, 657 bp, synthetic construct
  source 1..657: mol_type = other DNA
gacgtcgtgatgacccagtctcctctgtctctgcctgtgacacctggcgagcctgcctccatctcttgcagatcatctcagtccctggtgcactccaaccggaacacctacctgcactggtatctgcagaagcccggacagtctccccagctgctgatctacaaggtgtccaacagattctctggcgtgcccgacagattcagcggctctggctctggcaccgacttcaccctgaagatttccagagtggaagccgaggacgtgggcgtgtactactgctctcagaatacccacgtgccacctacctttggccagggcaccaagctggaaatcaagagaaccgtggccgctccttccgtgttcatcttcccaccatctgacgagcagctgaagtccggcacagcttctgtcgtgtgcctgctgaacaacttctaccctcgggaagccaaggtgcagtggaaggtggacaatgccctgcagtccggcaactcccaagagtctgtgaccgagcaggactccaaggactctacctacagcctgtcctccacactgaccctgtctaaggccgactacgagaagcacaaggtgtacgcctgtgaagtgacccaccagggcctgtctagccctgtgaccaagtctttcaaccggggcgagtgc